European Patent Specification EP 3 160 502 B1, published May 20, 2026. Title: Anti-IL4-IL13 Bispecific Antibodies. Applicant: Sanofi Esperet, Corinne Jagerschmidt, Alexandre Soubrane, Christina Subramaniam, Arun. The sequence listing filed with the application follows.

SEQUENCE LISTING (7 sequences)

SEQ ID NO: 1 - protein, 111 aa, Artificial Sequence
  humanized mouse/ mouse VL3 region
DIVLTQSPASLAVSLGQRATISCRASESVDSYGQSYMHWYQQKAGQPPKLLIYLASNLESGVPARFSGSGSRTDFTLTIDPVQAEDAATYYCQQNAEDSRTFGGGTKLEIK

SEQ ID NO: 2 - protein, 118 aa, Artificial Sequence
  humanized mouse/mouse VH2 region
EVQLKESGPGLVAPGGSLSITCTVSGFSLTDSSINWVRQPPGKGLEWLGMIWGDGRIDYADALKSRLSISKDSSKSQVFLEMTSLRTDDTATYYCARDGYFPYAMDFWGQGTSVTVSS

SEQ ID NO: 3 - protein, 108 aa, Artificial Sequence
  humanized mouse/mouse VL1 region
DIQMTQSPASLSVSVGDTITLTCHASQNIDVWLSWFQQKPGNIPKLLIYKASNLHTGVPSRFSGSGSGTGFTLTISSLQPEDIATYYCQQAHSYPFTFGGGTKLEIKR

SEQ ID NO: 4 - protein, 124 aa, Artificial Sequence
  humanized mouse/mouse VH1 region
QVQLQQSGPELVKPGASVKISCKASGYSFTSYWIHWIKQRPGQGLEWIGMIDPSDGETRLNQRFQGRATLTVDESTSTAYMQLRSPTSEDSAVYYCTRLKEYGNYDSFYFDVWGAGTLVTVSSA

SEQ ID NO: 5 - protein, 124 aa, Artificial Sequence
  humanized mouse/mouse VH2 region
QVQLQQSGPELVKPGASVKISCKASGYSFTSYWIHWIKQRPGQGLEWIGMIDASDGETRLNQRFQGRATLTVDESTSTAYMQLRSPTSEDSAVYYCTRLKEYGNYDSFYFDVWGAGTLVTVSSA

SEQ ID NO: 6 - protein, 10 aa, Artificial Sequence
  linker
GGGGSGGGGS

SEQ ID NO: 7 - DNA, 30 bp, Artificial Sequence
  primer
ggaggcggagggtccggaggcggaggatcc